European Patent Application EP 4 438 122 A2, published October 2, 2024. Title: RING-MODIFIED PROLINE SHORT PEPTIDE COMPOUND AND USE THEREOF. Applicant: Fujian Akeylink Biotechnology Co., Ltd. The sequence listing filed with the application follows.

SEQUENCE LISTING (1 sequence)

SEQ ID NO: 1 - protein, 13 aa, synthetic construct
  MOD_RES 1: note = modified with Dabcyl
  MOD_RES 13: note = modified with Edans
KTSAVLQSGFRKM